European Patent Specification EP 3 652 164 B1, published June 21, 2023. Title: PHENYLACETAMIDES AS INHIBITORS OF ROCK. Applicant: Bristol-Myers Squibb Company. The sequence listing filed with the application follows.

SEQUENCE LISTING (1 sequence)

SEQ ID NO: 1 - protein, 11 aa, Artificial Sequence
  Synthesized Peptide
  MISC_FEATURE: FITC-AHA at N Terminus attached at A1 - A11
  MISC_FEATURE: OH at C Terminus attached at A1 - A11
AKRRRLSSLRA